European Patent Specification EP 4 168 538 B1, published August 19, 2026. Title: COMBINING iPSC-DERIVED EFFECTOR CELL TYPES FOR IMMUNOTHERAPY USE. Applicant: Fate Therapeutics, Inc. The sequence listing filed with the application follows.

SEQUENCE LISTING (16 sequences)

SEQ ID NO: 1 - protein, 340 aa, Artificial Sequence
  CD64 domain-based construction
MWFLTTLLLWVPVDGQVDTTKAVITLQPPWVSVFQEETVTLHCEVLHLPGSSSTQWFLNGTATQTSTPSYRITSASVNDSGEYRCQRGLSGRSDPIQLEIHRGWLLLQVSSRVFTEGEPLALRCHAWKDKLVYNVLYYRNGKAFKFFHWNSNLTILKTNISHNGTYHCSGMGKHRYTSAGISVTVKELFPAPVLNASVTSPLLEGNLVTLSCETKLLLQRPGLQLYFSFYMGSKTLRGRNTSSEYQILTARREDSGLYWCEAATEDGNVLKRSPELELQVLGLQLPTPVWFHYQVSFCLVMVLLFAVDTGLYFSVKTNIRSSTRDWKDHKFKWRKDPQDK

SEQ ID NO: 2 - protein, 336 aa, Artificial Sequence
  CD64 exon-based construction
MWFLTTLLLWVPVDGQVDTTKAVITLQPPWVSVFQEETVTLHCEVLHLPGSSSTQWFLNGTATQTSTPSYRITSASVNDSGEYRCQRGLSGRSDPIQLEIHRGWLLLQVSSRVFTEGEPLALRCHAWKDKLVYNVLYYRNGKAFKFFHWNSNLTILKTNISHNGTYHCSGMGKHRYTSAGISVTVKELFPAPVLNASVTSPLLEGNLVTLSCETKLLLQRPGLQLYFSFYMGSKTLRGRNTSSEYQILTARREDSGLYWCEAATEDGNVLKRSPELELQVLGLFFPPGYQVSFCLVMVLLFAVDTGLYFSVKTNIRSSTRDWKDHKFKWRKDPQDK

SEQ ID NO: 3 - protein, 335 aa, Artificial Sequence
  CD64 exon-based construction
MWFLTTLLLWVPVDGQVDTTKAVITLQPPWVSVFQEETVTLHCEVLHLPGSSSTQWFLNGTATQTSTPSYRITSASVNDSGEYRCQRGLSGRSDPIQLEIHRGWLLLQVSSRVFTEGEPLALRCHAWKDKLVYNVLYYRNGKAFKFFHWNSNLTILKTNISHNGTYHCSGMGKHRYTSAGISVTVKELFPAPVLNASVTSPLLEGNLVTLSCETKLLLQRPGLQLYFSFYMGSKTLRGRNTSSEYQILTARREDSGLYWCEAATEDGNVLKRSPELELQVLGFFPPGYQVSFCLVMVLLFAVDTGLYFSVKTNIRSSTRDWKDHKFKWRKDPQDK

SEQ ID NO: 4 - DNA, 1032 bp, Artificial Sequence
  CD64 domain-based construction (encoding SEQ ID NO. 1)
cttggagacaacatgtggttcttgacaactctgctcctttgggttccagttgatgggcaagtggacaccacaaaggcagtgatcactttgcagcctccatgggtcagcgtgttccaagaggaaaccgtaaccttgcattgtgaggtgctccatctgcctgggagcagctctacacagtggtttctcaatggcacagccactcagacctcgacccccagctacagaatcacctctgccagtgtcaatgacagtggtgaatacaggtgccagagaggtctctcagggcgaagtgaccccatacagctggaaatccacagaggctggctactactgcaggtctccagcagagtcttcacggaaggagaacctctggccttgaggtgtcatgcgtggaaggataagctggtgtacaatgtgctttactatcgaaatggcaaagcctttaagtttttccactggaattctaacctcaccattctgaaaaccaacataagtcacaatggcacctaccattgctcaggcatgggaaagcatcgctacacatcagcaggaatatctgtcactgtgaaagagctatttccagctccagtgctgaatgcatctgtgacatccccactcctggaggggaatctggtcaccctgagctgtgaaacaaagttgctcttgcagaggcctggtttgcagctttacttctccttctacatgggcagcaagaccctgcgaggcaggaacacatcctctgaataccaaatactaactgctagaagagaagactctgggttatactggtgcgaggctgccacagaggatggaaatgtccttaagcgcagccctgagttggagcttcaagtgcttggcctccagttaccaactcctgtctggtttcattaccaagtctctttctgcttggtgatggtactcctttttgcagtggacacaggactatatttctctgtgaagacaaacattcgaagctcaacaagagactggaaggaccataaatttaaatggagaaaggaccctcaagacaaa

SEQ ID NO: 5 - DNA, 1020 bp, Artificial Sequence
  CD64 exon-based construction (encoding SEQ ID NO. 2)
cttggagacaacatgtggttcttgacaactctgctcctttgggttccagttgatgggcaagtggacaccacaaaggcagtgatcactttgcagcctccatgggtcagcgtgttccaagaggaaaccgtaaccttgcattgtgaggtgctccatctgcctgggagcagctctacacagtggtttctcaatggcacagccactcagacctcgacccccagctacagaatcacctctgccagtgtcaatgacagtggtgaatacaggtgccagagaggtctctcagggcgaagtgaccccatacagctggaaatccacagaggctggctactactgcaggtctccagcagagtcttcacggaaggagaacctctggccttgaggtgtcatgcgtggaaggataagctggtgtacaatgtgctttactatcgaaatggcaaagcctttaagtttttccactggaattctaacctcaccattctgaaaaccaacataagtcacaatggcacctaccattgctcaggcatgggaaagcatcgctacacatcagcaggaatatctgtcactgtgaaagagctatttccagctccagtgctgaatgcatctgtgacatccccactcctggaggggaatctggtcaccctgagctgtgaaacaaagttgctcttgcagaggcctggtttgcagctttacttctccttctacatgggcagcaagaccctgcgaggcaggaacacatcctctgaataccaaatactaactgctagaagagaagactctgggttatactggtgcgaggctgccacagaggatggaaatgtccttaagcgcagccctgagttggagcttcaagtgcttggtttgttctttccacctgggtaccaagtctctttctgcttggtgatggtactcctttttgcagtggacacaggactatatttctctgtgaagacaaacattcgaagctcaacaagagactggaaggaccataaatttaaatggagaaaggaccctcaagacaaa

SEQ ID NO: 6 - DNA, 1005 bp, Artificial Sequence
  CD64 exon-based construction (encoding SEQ ID NO. 3)
atgtggttcttgacaactctgctcctttgggttccagttgatgggcaagtggacaccacaaaggcagtgatcactttgcagcctccatgggtcagcgtgttccaagaggaaaccgtaaccttgcactgtgaggtgctccatctgcctgggagcagctctacacagtggtttctcaatggcacagccactcagacctcgacccccagctacagaatcacctctgccagtgtcaatgacagtggtgaatacaggtgccagagaggtctctcagggcgaagtgaccccatacagctggaaatccacagaggctggctactactgcaggtctccagcagagtcttcacggaaggagaacctctggccttgaggtgtcatgcgtggaaggataagctggtgtacaatgtgctttactatcgaaatggcaaagcctttaagtttttccactggaactctaacctcaccattctgaaaaccaacataagtcacaatggcacctaccattgctcaggcatgggaaagcatcgctacacatcagcaggaatatctgtcactgtgaaagagctatttccagctccagtgctgaatgcatctgtgacatccccactcctggaggggaatctggtcaccctgagctgtgaaacaaagttgctcttgcagaggcctggtttgcagctttacttctccttctacatgggcagcaagaccctgcgaggcaggaacacatcctctgaataccaaatactaactgctagaagagaagactctgggttatactggtgcgaggctgccacagaggatggaaatgtccttaagcgcagccctgagttggagcttcaagtgcttggcttctttccacctgggtaccaagtctctttctgcttggtgatggtactcctttttgcagtggacacaggactatatttctctgtgaagacaaacattcgaagctcaacaagagactggaaggaccataaatttaaatggagaaaggaccctcaagacaaa

SEQ ID NO: 7 - protein, 153 aa, Artificial Sequence
  CD28 co-stim + CD3-zeta-ITAM construct
RSKRSRLLHSDYMNMTPRRPGPTRKHYQPYAPPRDFAAYRSRVKFSRSADAPAYQQGQNQLYNELNLGRREEYDVLDKRRGRDPEMGGKPRRKNPQEGLFNELQKDKMAEAFSEIGMKGERRRGKGHDGLFQGLSTATKDTFDALHMQALPPR

SEQ ID NO: 8 - protein, 219 aa, Artificial Sequence
  CD28 hinge + CD28 TM + CD28 co-stim + CD3-zeta-ITAM construct
IEVMYPPPYLDNEKSNGTIIHVKGKHLCPSPLFPGPSKPFWVLVVVGGVLACYSLLVTVAFIIFWVRSKRSRLLHSDYMNMTPRRPGPTRKHYQPYAPPRDFAAYRSRVKFSRSADAPAYQQGQNQLYNELNLGRREEYDVLDKRRGRDPEMGGKPRRKNPQEGLFNELQKDKMAEAFSEIGMKGERRRGKGHDGLFQGLSTATKDTFDALHMQALPPR

SEQ ID NO: 9 - protein, 263 aa, Artificial Sequence
  NKG2D TM + 2B4 + CD3-zeta construct
SNLFVASWIAVMIIFRIGMAVAIFCCFFFPSWRRKRKEKQSETSPKEFLTIYEDVKDLKTRRNHEQEQTFPGGGSTIYSMIQSQSSAPTSQEPAYTLYSLIQPSRKSGSRKRNHSPSFNSTIYEVIGKSQPKAQNPARLSRKELENFDVYSRVKFSRSADAPAYKQGQNQLYNELNLGRREEYDVLDKRRGRDPEMGGKPRRKNPQEGLYNELQKDKMAEAYSEIGMKGERRRGKGHDGLYQGLSTATKDTYDALHMQALPPR

SEQ ID NO: 10 - protein, 308 aa, Artificial Sequence
  CD8 hinge + NKG2D TM + 2B4 + CD3-zeta construct
TTTPAPRPPTPAPTIASQPLSLRPEACRPAAGGAVHTRGLDFACDSNLFVASWIAVMIIFRIGMAVAIFCCFFFPSWRRKRKEKQSETSPKEFLTIYEDVKDLKTRRNHEQEQTFPGGGSTIYSMIQSQSSAPTSQEPAYTLYSLIQPSRKSGSRKRNHSPSFNSTIYEVIGKSQPKAQNPARLSRKELENFDVYSRVKFSRSADAPAYKQGQNQLYNELNLGRREEYDVLDKRRGRDPEMGGKPRRKNPQEGLYNELQKDKMAEAYSEIGMKGERRRGKGHDGLYQGLSTATKDTYDALHMQALPPR

SEQ ID NO: 11 - protein, 414 aa, Artificial Sequence
  a construct mimicking trans-presentation of IL15 (Design 2)
MDWTWILFLVAAATRVHSGIHVFILGCFSAGLPKTEANWVNVISDLKKIEDLIQSMHIDATLYTESDVHPSCKVTAMKCFLLELQVISLESGDASIHDTVENLIILANNSLSSNGNVTESGCKECEELEEKNIKEFLQSFVHIVQMFINTSSGGGSGGGGSGGGGSGGGGSGGGSLQITCPPPMSVEHADIWVKSYSLYSRERYICNSGFKRKAGTSSLTECVLNKATNVAHWTTPSLKCIRDPALVHQRPAPPSTVTTAGVTPQPESLSPSGKEPAASSPSSNNTAATTAAIVPGSQLMPSKSPSTGTTEISSHESSHGTPSQTTAKNWELTASASHQPPGVYPQGHSDTTVAISTSTVLLCGLSAVSLLACYLKSRQTPPLASVEMEAMEALPVTWGTSSRDEDLENCSHHL

SEQ ID NO: 12 - DNA, 1242 bp, Artificial Sequence
  exemplary DNA sequence encoding the amino acid sequence of SEQ ID NO: 11
atggactggacctggattctgttcctggtcgcggctgcaacgcgagtccatagcggtatccatgtttttattcttgggtgtttttctgctgggctgcctaagaccgaggccaactgggtaaatgtcatcagtgacctcaagaaaatagaagaccttatacaaagcatgcacattgatgctactctctacactgagtcagatgtacatccctcatgcaaagtgacggccatgaaatgtttcctcctcgaacttcaagtcatatctctggaaagtggcgacgcgtccatccacgacacggtcgaaaacctgataatactcgctaataatagtctctcttcaaatggtaacgtaaccgagtcaggttgcaaagagtgcgaagagttggaagaaaaaaacataaaggagttcctgcaaagtttcgtgcacattgtgcagatgttcattaatacctctagcggcggaggatcaggtggcggtggaagcggaggtggaggctccggtggaggaggtagtggcggaggttctcttcaaataacttgtcctccaccgatgtccgtagaacatgcggatatttgggtaaaatcctatagcttgtacagccgagagcggtatatctgcaacagcggcttcaagcggaaggccggcacaagcagcctgaccgagtgcgtgctgaacaaggccaccaacgtggcccactggaccacccctagcctgaagtgcatcagagatcccgccctggtgcatcagcggcctgcccctccaagcacagtgacaacagctggcgtgaccccccagcctgagagcctgagcccttctggaaaagagcctgccgccagcagccccagcagcaacaatactgccgccaccacagccgccatcgtgcctggatctcagctgatgcccagcaagagccctagcaccggcaccaccgagatcagcagccacgagtctagccacggcaccccatctcagaccaccgccaagaactgggagctgacagccagcgcctctcaccagcctccaggcgtgtaccctcagggccacagcgataccacagtggccatcagcacctccaccgtgctgctgtgtggactgagcgccgtgtcactgctggcctgctacctgaagtccagacagacccctccactggccagcgtggaaatggaagccatggaagcactgcccgtgacctggggcaccagctccagagatgaggatctggaaaactgctcccaccacctg

SEQ ID NO: 13 - protein, 379 aa, Artificial Sequence
  a construct mimicking trans-presentation of IL15 (Design 3)
MDWTWILFLVAAATRVHSGIHVFILGCFSAGLPKTEANWVNVISDLKKIEDLIQSMHIDATLYTESDVHPSCKVTAMKCFLLELQVISLESGDASIHDTVENLIILANNSLSSNGNVTESGCKECEELEEKNIKEFLQSFVHIVQMFINTSSGGGSGGGGSGGGGSGGGGSGGGSLQITCPPPMSVEHADIWVKSYSLYSRERYICNSGFKRKAGTSSLTECVLNKATNVAHWTTPSLKCIRDPALVHQRPAPPSTVTTAGVTPQPESLSPSGKEPAASSPSSNNTAATTAAIVPGSQLMPSKSPSTGTTEISSHESSHGTPSQTTAKNWELTASASHQPPGVYPQGHSDTTVAISTSTVLLCGLSAVSLLACYLKSRQ

SEQ ID NO: 14 - DNA, 1140 bp, Artificial Sequence
  exemplary nucleic acid sequence encoding the amino acid sequence of SEQ ID NO: 13
atggactggacctggattctgttcctggtcgcggctgcaacgcgagtccatagcggtatccatgtttttattcttgggtgtttttctgctgggctgcctaagaccgaggccaactgggtaaatgtcatcagtgacctcaagaaaatagaagaccttatacaaagcatgcacattgatgctactctctacactgagtcagatgtacatccctcatgcaaagtgacggccatgaaatgtttcctcctcgaacttcaagtcatatctctggaaagtggcgacgcgtccatccacgacacggtcgaaaacctgataatactcgctaataatagtctctcttcaaatggtaacgtaaccgagtcaggttgcaaagagtgcgaagagttggaagaaaaaaacataaaggagttcctgcaaagtttcgtgcacattgtgcagatgttcattaatacctctagcggcggaggatcaggtggcggtggaagcggaggtggaggctccggtggaggaggtagtggcggaggttctcttcaaataacttgtcctccaccgatgtccgtagaacatgcggatatttgggtaaaatcctatagcttgtacagccgagagcggtatatctgcaacagcggcttcaagcggaaggccggcacaagcagcctgaccgagtgcgtgctgaacaaggccaccaacgtggcccactggaccacccctagcctgaagtgcatcagagatcccgccctggtgcatcagcggcctgcccctccaagcacagtgacaacagctggcgtgaccccccagcctgagagcctgagcccttctggaaaagagcctgccgccagcagccccagcagcaacaatactgccgccaccacagccgccatcgtgcctggatctcagctgatgcccagcaagagccctagcaccggcaccaccgagatcagcagccacgagtctagccacggcaccccatctcagaccaccgccaagaactgggagctgacagccagcgcctctcaccagcctccaggcgtgtaccctcagggccacagcgataccacagtggccatcagcacctccaccgtgctgctgtgtggactgagcgccgtgtcactgctggcctgctacctgaagtccagacagtga

SEQ ID NO: 15 - protein, 242 aa, Artificial Sequence
  a construct mimicking trans-presentation of IL15 (Design 4)
MDWTWILFLVAAATRVHSGIHVFILGCFSAGLPKTEANWVNVISDLKKIEDLIQSMHIDATLYTESDVHPSCKVTAMKCFLLELQVISLESGDASIHDTVENLIILANNSLSSNGNVTESGCKECEELEEKNIKEFLQSFVHIVQMFINTSSGGGSGGGGSGGGGSGGGGSGGGSLQITCPPPMSVEHADIWVKSYSLYSRERYICNSGFKRKAGTSSLTECVLNKATNVAHWTTPSLKCIR

SEQ ID NO: 16 - DNA, 726 bp, Artificial Sequence
  exemplary nucleic acid sequence encoding the amino acid sequence of SEQ ID NO: 15
atggactggacctggattctgttcctggtcgcggctgcaacgcgagtccatagcggtatccatgtttttattcttgggtgtttttctgctgggctgcctaagaccgaggccaactgggtaaatgtcatcagtgacctcaagaaaatagaagaccttatacaaagcatgcacattgatgctactctctacactgagtcagatgtacatccctcatgcaaagtgacggccatgaaatgtttcctcctcgaacttcaagtcatatctctggaaagtggcgacgcgtccatccacgacacggtcgaaaacctgataatactcgctaataatagtctctcttcaaatggtaacgtaaccgagtcaggttgcaaagagtgcgaagagttggaagaaaaaaacataaaggagttcctgcaaagtttcgtgcacattgtgcagatgttcattaatacctctagcggcggaggatcaggtggcggtggaagcggaggtggaggctccggtggaggaggtagtggcggaggttctcttcaaataacttgtcctccaccgatgtccgtagaacatgcggatatttgggtaaaatcctatagcttgtacagccgagagcggtatatctgcaacagcggcttcaagcggaaggccggcacaagcagcctgaccgagtgcgtgctgaacaaggccaccaacgtggcccactggaccacccctagcctgaagtgcatcaga